European Patent Specification EP 3 711 778 B1, published May 8, 2024. Title: METHODS AND COMPOSITIONS FOR INCREASING ARYLSULFATASE A ACTIVITY IN THE CNS. Applicant: ARMAGEN TECHNOLOGIES, INC. Application To be Assigned. The sequence listing filed with the application follows.

SEQUENCE LISTING (12 sequences)

SEQ ID NO: 1 - protein, 10 aa, Artificial sequence
  Synthetic protein
GYTFTNYDIH

SEQ ID NO: 2 - protein, 17 aa, Artificial sequence
  Synthetic protein
WIYPGDGSTKYNEKFKG

SEQ ID NO: 3 - protein, 4 aa, Artificial sequence
  Synthetic protein
EWAY

SEQ ID NO: 4 - protein, 11 aa, Artificial sequence
  Synthetic protein
RASQDIGGNLY

SEQ ID NO: 5 - protein, 7 aa, Artificial sequence
  Synthetic protein
ATSSLDS

SEQ ID NO: 6 - protein, 9 aa, Artificial sequence
  Synthetic protein
LQYSSSPWT

SEQ ID NO: 7 - protein, 462 aa, Artificial sequence
  Synthetic protein
MDWTWRVFCLLAVAPGAHSQVQLQQSGPELVKPGALVKISCKASGYTFTNYDIHWVKQRPGQGLEWIGWIYPGDGSTKYNEKFKGKATLTADKSSSTAYMHLSSLTSEKSAVYFCAREWAYWGQGTLVTVSAASTKGPSVFPLAPSSKSTSGGTAALGCLVKDYFPEPVTVSWNSGALTSGVHTFPAVLQSSGLYSLSSVVTVPSSSLGTQTYICNVNHKPSNTKVDKKVEPKSCDKTHTCPPCPAPELLGGPSVFLFPPKPKDTLMISRTPEVTCVVVDVSHEDPEVKFNWYVDGVEVHNAKTKPREEQYNSTYRVVSVLTVLHQDWLNGKEYKCKVSNKALPAPIEKTISKAKGQPREPQVYTLPPSRDELTKNQVSLTCLVKGFYPSDIAVEWESNGQPENNYKTTPPVLDSDGSFFLYSKLTVDKSRWQQGNVFSCSVMHEALHNHYTQKSLSLSPGK

SEQ ID NO: 8 - protein, 234 aa, Artificial sequence
  Synthetic protein
METPAQLLFLLLLWLPDTTGDIQMTQSPSSLSASLGERVSLTCRASQDIGGNLYWLQQGPDGTIKRLIYATSSLDSGVPKRFSGSRSGSDYSLTISSLESEDFVDYYCLQYSSSPWTFGGGTKMEIKRTVAAPSVFIFPPSDEQLKSGTASVVCLLNNFYPREAKVQWKVDNALQSGNSQESVTEQDSKDSTYSLSSTLTLSKADYEKHKVYACEVTHQGLSSPVTKSFNRGEC

SEQ ID NO: 9 - protein, 489 aa, Artificial sequence
  Synthetic protein
RPPNIVLIFADDLGYGDLGCYGHPSSTTPNLDQLAAGGLRFTDFYVPVSLCTPSRAALLTGRLPVRMGMYPGVLVPSSRGGLPLEEVTVAEVLAARGYLTGMAGKWHLGVGPEGAFLPPHQGFHRFLGIPYSHDQGPCQNLTCFPPATPCDGGCDQGLVPIPLLANLSVEAQPPWLPGLEARYMAFAHDLMADAQRQDRPFFLYYASHHTHYPQFSGQSFAERSGRGPFGDSLMELDAAVGTLMTAIGDLGLLEETLVIFTADNGPETMRMSRGGCSGLLRCGKGTTYEGGVREPALAFWPGHIAPGVTHELASSLDLLPTLAALAGAPLPNVTLDGFDLSPLLLGTGKSPRQSLFFYPSYPDEVRGVFAVRSGKYKAHFFTQGSAHSDTTADPACHASSSLTAHEPPLLYDLSKDPGENYNLLGGVAGATPEVLQALKQLQLLKAQLDAAVTFGPSQVARGEDPALQICCHPGCTPRPACCHCPDPHA

SEQ ID NO: 10 - protein, 953 aa, Artificial sequence [sequence omitted]

SEQ ID NO: 11 - DNA, 22 bp, Artificial sequence
  Synthetic DNA
cccgtccgcccaacatcgtgct

SEQ ID NO: 12 - DNA, 24 bp, Artificial sequence
  Synthetic DNA
tcaggcatggggatctgggcaatg